European Patent Application EP 4 640 696 A1, published October 29, 2025. Title: 변이체 폴리펩티드 및 이를 이용한 L-글루탐산 생산 방법. Applicant: CJ CheilJedang Corporation. The sequence listing filed with the application follows.

SEQUENCE LISTING (24 sequences)

SEQ ID NO: 1 - protein, 494 aa, Corynebacterium glutamicum
MISETLQAQAPTKTQRWAFLAVISGGLFLIGVDNSILYTALPLLREQLAATETQALWIINAYPLLMAGLLLGTGTLGDKIGHRRMFLMGLSIFGIASLGAAFAPTAWALVAARAFLGIGAATMMPATLALIRITFEDERERNTAIGIWGSVAILGAAAGPIIGGALLEFFWWGSVFLINVPVAVIALIATLFVAPANIANPSKHWDFLSSFYALLTLAGLIVTIKESVNTARHLPLLVGAIILLIIGAVLFSSRQKKIEEPLLDLSLFRNRLFLGGVVAAGMAMFTVSGLEMTTSQRFQLSVGFTPLEAGLLMIPAALGSFPMSIIGGANLHRWGFKPLISGGFLATAVGIALCIWGATHTDGLPFFIAGLFFMGAGAGSVMSVSSTAIIGSAPVRKAGMASSIEEVSYEFGTLLSVAILGSLFPFFYSLHAPAEVADNFSAGVHHAIYGDAARASLDTAYINVLIIALVCAVAAALISSYLFRGNPKGANNAH

SEQ ID NO: 2 - DNA, 1485 bp, Corynebacterium glutamicum
  source 1..1485: mol_type = genomic DNA
atgatttcagaaactttgcaggcgcaagcgcctacgaaaacccaacgttgggctttcctcgctgttatcagcggtggtctctttctgatcggtgtagacaactcaatcctctacaccgcactccccctgctgcgtgaacaactcgcagccactgaaacccaagcgttgtggatcatcaacgcatatcccctgctcatggcgggtcttcttttgggtaccggcactttgggtgacaaaatcggccaccgccggatgttcctcatgggcttgagcattttcggaatcgcttcacttggcgctgcgtttgctccaactgcgtgggctcttgttgctgcgagagctttccttggcatcggtgcggcgacgatgatgcccgcaaccttggctctgatccgcattacgtttgaagatgaacgcgaacggaacaccgcgattggcatttggggttctgtggcaattcttggcgcggcggcaggtccgatcattggtggtgcgctgttggaattcttctggtggggttcggttttcctcattaacgttccggtggctgttatcgcgttgatcgctacgctttttgtggcgccggccaatatcgcgaatccgtccaagcactgggatttcttatcctcgttctatgcattgcttacccttgcaggtttgattgtcaccatcaaagaatcggtaaacactgcacgtcatctgccactgcttgtaggtgccatcatcttgcttatcattggtgcggtgttgtttagcagtcgtcagaagaagatcgaggagccacttctagatctgtcgttgttccgtaatcgccttttcttaggcggtgtggttgctgcgggcatggcgatgtttactgtgtccggtttggaaatgactacctcgcagcgtttccagttgtctgtgggtttcactccacttgaggctggtttgctcatgatcccagctgcattgggtagcttcccgatgtctattatcggtggtgcaaacttgcatcgttggggcttcaaaccgctgatcagtggtggtttccttgccacggcagtcggcatcgccctgtgtatttggggcgcgactcatactgatggtttgccgtttttcatcgcgggtctgttcttcatgggcgcgggtgctggttcggtaatgtctgtgtcttccactgcgattatcggttccgcgccggtgcgtaaggctggcatggcgtcgtcgatcgaagaggtctcttatgagttcggcacgctgttgtctgtcgcgattttgggtagcttgttcccattcttctactcgctgcatgccccggcagaggttgcggataacttctcggcgggtgttcaccacgcgatttatggcgatgcggcgcgtgcatctttggacaccgcatacattaacgtgttgatcattgccctagtatgcgcagtagcggctgctctgatcagcagttaccttttccgcggaaatccgaagggagccaataatgcgcactag

SEQ ID NO: 3 - protein, 494 aa, synthetic construct
MISETLQAQAPTKTQRWAFLAVISGGLFLIGVDNSILYTALPLLREQLAATETQALWIINAYPLLMAGLLLGTGTLGDKIGHRRMFLMGLSIFGIASLGAAFAPTAWALVAARAFLGIGAATMMPATLALIRITFEDERERNTAIGIWGSVAILGAAAGPIIGGALLEFFWWGSVFLINVPVAVIALIATLFVAPANIANPSKHWDFLSSFYALLTLAGLIVTIKESVNTARHLPLLVGAIILLIIGAVLFSSRQKKIEEPLLDLSLFRNRLFLGGVVAAGMAMFTVSGLEMTTSQRFQLSVGFTPLEAGLLMIPAALGSFPMSIIGGANLHRWGFKPLISGGFLATAVGNALCIWGATHTDGLPFFIAGLFFMGAGAGSVMSVSSTAIIGSAPVRKAGMASSIEEVSYEFGTLLSVAILGSLFPFFYSLHAPAEVADNFSAGVHHAIYGDAARASLDTAYINVLIIALVCAVAAALISSYLFRGNPKGANNAH

SEQ ID NO: 4 - DNA, 1485 bp, synthetic construct
  source 1..1485: mol_type = other DNA
atgatttcagaaactttgcaggcgcaagcgcctacgaaaacccaacgttgggctttcctcgctgttatcagcggtggtctctttctgatcggtgtagacaactcaatcctctacaccgcactccccctgctgcgtgaacaactcgcagccactgaaacccaagcgttgtggatcatcaacgcatatcccctgctcatggcgggtcttcttttgggtaccggcactttgggtgacaaaatcggccaccgccggatgttcctcatgggcttgagcattttcggaatcgcttcacttggcgctgcgtttgctccaactgcgtgggctcttgttgctgcgagagctttccttggcatcggtgcggcgacgatgatgcccgcaaccttggctctgatccgcattacgtttgaagatgaacgcgaacggaacaccgcgattggcatttggggttctgtggcaattcttggcgcggcggcaggtccgatcattggtggtgcgctgttggaattcttctggtggggttcggttttcctcattaacgttccggtggctgttatcgcgttgatcgctacgctttttgtggcgccggccaatatcgcgaatccgtccaagcactgggatttcttatcctcgttctatgcattgcttacccttgcaggtttgattgtcaccatcaaagaatcggtaaacactgcacgtcatctgccactgcttgtaggtgccatcatcttgcttatcattggtgcggtgttgtttagcagtcgtcagaagaagatcgaggagccacttctagatctgtcgttgttccgtaatcgccttttcttaggcggtgtggttgctgcgggcatggcgatgtttactgtgtccggtttggaaatgactacctcgcagcgtttccagttgtctgtgggtttcactccacttgaggctggtttgctcatgatcccagctgcattgggtagcttcccgatgtctattatcggtggtgcaaacttgcatcgttggggcttcaaaccgctgatcagtggtggtttccttgccacggcagtcggcaacgccctgtgtatttggggcgcgactcatactgatggtttgccgtttttcatcgcgggtctgttcttcatgggcgcgggtgctggttcggtaatgtctgtgtcttccactgcgattatcggttccgcgccggtgcgtaaggctggcatggcgtcgtcgatcgaagaggtctcttatgagttcggcacgctgttgtctgtcgcgattttgggtagcttgttcccattcttctactcgctgcatgccccggcagaggttgcggataacttctcggcgggtgttcaccacgcgatttatggcgatgcggcgcgtgcatctttggacaccgcatacattaacgtgttgatcattgccctagtatgcgcagtagcggctgctctgatcagcagttaccttttccgcggaaatccgaagggagccaataatgcgcactag

SEQ ID NO: 5 - protein, 160 aa, Corynebacterium glutamicum
LSRAAAEIALMEGPEAFTVAAIAAAAGVSPRTFHNYFPSREDALVQFVVIRVQELTDQLYEFPTSVPPRDAIEQLVINQLRDGDDAMDSFSAMFRIGEILENLDPIKCVIDKERLIAPLLEFMVERDKDLDKFDAATLIHLHAAAIATSLHTFYQAPEPR

SEQ ID NO: 6 - DNA, 537 bp, Corynebacterium glutamicum
  source 1..537: mol_type = genomic DNA
ttgtcacgtgctgctgcggagatcgccttgatggaaggccctgaggcgttcacggttgcggccattgcagctgcagccggggtctccccccggacttttcataactacttcccttctcgggaagacgcattggtgcaatttgtggtcattcgcgttcaggaactcacggatcagctatacgagtttcctacaagcgtgcccccacgagatgccattgaacaattggtgatcaaccaattgcgggatggcgatgacgctatggattctttcagcgcaatgtttcgaatcggtgagatccttgaaaatcttgaccccatcaagtgtgttatcgataaggagcgactcattgctccgttgcttgagttcatggttgaacgtgacaaagaccttgacaagttcgatgcggcaactctgatccatttgcatgcagcggcaattgcaacctcgctgcatacgttttaccaagctcccgagccccgggacatagaagatggagtcgcattgatccgtcgggcatgcgcctggattaagaaataa

SEQ ID NO: 7 - protein, 178 aa, synthetic construct
LSRAAAEIALMEGPEAFTVAAIAAAAGVSPRTFHNYFPSREDALVQFVVIRVQELTDQLYEFPTSVPPRDAIEQLVINQLRDGDDAMDSFSAMFRIGEILENLDLIKCVIDKERLIAPLLEFMVERDKDLDKFDAATLIHLHAAAIATSLHTFYQAPEPRDIEDGVALIRRACAWIKK

SEQ ID NO: 8 - DNA, 537 bp, synthetic construct
  source 1..537: mol_type = other DNA
ttgtcacgtgctgctgcggagatcgccttgatggaaggccctgaggcgttcacggttgcggccattgcagctgcagccggggtctccccccggacttttcataactacttcccttctcgggaagacgcattggtgcaatttgtggtcattcgcgttcaggaactcacggatcagctatacgagtttcctacaagcgtgcccccacgagatgccattgaacaattggtgatcaaccaattgcgggatggcgatgacgctatggattctttcagcgcaatgtttcgaatcggtgagatccttgaaaatcttgacctcatcaagtgtgttatcgataaggagcgactcattgctccgttgcttgagttcatggttgaacgtgacaaagaccttgacaagttcgatgcggcaactctgatccatttgcatgcagcggcaattgcaacctcgctgcatacgttttaccaagctcccgagccccgggacatagaagatggagtcgcattgatccgtcgggcatgcgcctggattaagaaataa

SEQ ID NO: 9 - protein, 432 aa, Corynebacterium glutamicum
MSNVGKPRTAQEIQQDWDTNPRWNGITRDYTADQVADLQGSVIEEHTLARRGSEILWDAVTQEGDGYINALGALTGNQAVQQVRAGLKAVYLSGWQVAGDANLSGHTYPDQSLYPANSVPSVVRRINNALLRSDEIARSEGDTSVDNWVVPIVADGEAGFGGALNVYELQKAMIAAGAAGTHWEDQLASEKKCGHLGGKVLIPTQQHIRTLNSARLAADVANTPTVVIARTDAEAATLITSDVDERDQPFITGERTAEGYYHVKNGLEPCIARAKSYAPYADMIWMETGTPDLELAKKFAEGVRSEFPDQLLSYNCSPSFNWSAHLEADEIAKFQKELGAMGFKFQFITLAGFHSLNYGMFDLAYGYAREGMTSFVDLQNREFKAAEERGFTAVKHQREVGAGYFDQIATTVDPNSSTTALKGSTEEGQFHN

SEQ ID NO: 10 - DNA, 1160 bp, Corynebacterium glutamicum
  source 1..1160: mol_type = genomic DNA
atgtcaaacgttggaaagccacgtaccgcacaggaaatccagcaggattgggacaccaaccctcgttggaacggcatcacccgcgactacaccgcagaccaggtagctgatctgcagggttccgtcatcgaggagcacactcttgctcgccgcggctcagagatcctctgggacgcagtcacccaggaaggtgacggatacatcaacgcgcttggcgcactcaccggtaaccaggctgttcagcaggttcgtgcaggcctgaaggctgtctacctgtccggttggcaggttgcaggtgacgccaacctctccggccacacctaccctgaccagtccctctacccagcgaactccgttccaagcgtcgttcgtcgcatcaacaacgcactgctgcgttccgatgaaatcgcacgctccgaaggcgacacctccgttgacaactgggttgtcccaatcgtcgcggacggcgaagctggcttcggtggagcactcaacgtctacgaactccagaaggcaatgatcgcagctggcgctgcaggcacccactgggaagaccagctcgcttctgaaaagaagtgtggccacctcggcggcaaggttctgatcccaacccagcagcacatccgcaccctgaactctgcccgccttgcagcagacgttgcaaacaccccaactgttgttatcgcacgtaccgacgctgaggcagcaaccctgatcacctctgacgttgatgagcgcgaccaaccattcatcaccggtgagcgcaccgcagaaggctactaccacgtcaagaatggtctcgagccatgtatcgcacgtgcaaagtcctacgcaccatacgcagatatgatctggatggagaccggcacccctgacctggagctcgctaagaagttcgctgaaggcgttcgctctgagttcccagaccagctgctgtcctacaactgctccccatccttcaactggtctgcacacctcgaggcagatgagatcgctaagttccagaaggaactgggagctatgggcttcaagttccagttcatcaccctcgcaggcttccactccctcaactacggcatgttcgacctggcttacggatacgctcgcgaaggcatgacctccttcgttgacctgcagaaccgtgagttcaaggcagctga

SEQ ID NO: 11 - protein, 421 aa, synthetic construct
MSNVGKPRTAQEIQQDWDTNPRWNGITRDYTADQVADLQGSVIEEHTLARRGSEILWDAVTQEGDGYINALGALTGNQAVQQVRAGLKAVYLSGWQVAGDANLSGHTYPDQSLYPANSVPSVVRRINNALLRSDEIARSEGDTSVDNWVVPIVADGEAGFGGALNVYELQKAMIAAGAAGTHWEDQLASEKKCGHLGGKVLIPTQQHIRTLNSARLAADVANTPTVVIARTDAEAATLITSDVDERDQPFITGERTAEGYYHVKNGLEPCIARAKSYAPYADMIWMETGTPDLELAKKFAEGVRSEFPDQLLSYNCSPSFNWSAHLEADEIAKFQFITLAGFHSLNYGMFDLAYGYAREGMTSFVDLQNREFKAAEERGFTAVKHQREVGAGYFDQIATTVDPNSSTTALKGSTEEGQFHN

SEQ ID NO: 12 - DNA, 1266 bp, synthetic construct
  source 1..1266: mol_type = other DNA
atgtcaaacgttggaaagccacgtaccgcacaggaaatccagcaggattgggacaccaaccctcgttggaacggcatcacccgcgactacaccgcagaccaggtagctgatctgcagggttccgtcatcgaggagcacactcttgctcgccgcggctcagagatcctctgggacgcagtcacccaggaaggtgacggatacatcaacgcgcttggcgcactcaccggtaaccaggctgttcagcaggttcgtgcaggcctgaaggctgtctacctgtccggttggcaggttgcaggtgacgccaacctctccggccacacctaccctgaccagtccctctacccagcgaactccgttccaagcgtcgttcgtcgcatcaacaacgcactgctgcgttccgatgaaatcgcacgctccgaaggcgacacctccgttgacaactgggttgtcccaatcgtcgcggacggcgaagctggcttcggtggagcactcaacgtctacgaactccagaaggcaatgatcgcagctggcgctgcaggcacccactgggaagaccagctcgcttctgaaaagaagtgtggccacctcggcggcaaggttctgatcccaacccagcagcacatccgcaccctgaactctgcccgccttgcagcagacgttgcaaacaccccaactgttgttatcgcacgtaccgacgctgaggcagcaaccctgatcacctctgacgttgatgagcgcgaccaaccattcatcaccggtgagcgcaccgcagaaggctactaccacgtcaagaatggtctcgagccatgtatcgcacgtgcaaagtcctacgcaccatacgcagatatgatctggatggagaccggcacccctgacctggagctcgctaagaagttcgctgaaggcgttcgctctgagttcccagaccagctgctgtcctacaactgctccccatccttcaactggtctgcacacctcgaggcagatgagatcgctaagttccagttcatcaccctcgcaggcttccactccctcaactacggcatgttcgacctggcttacggatacgctcgcgaaggcatgacctccttcgttgacctgcagaaccgtgagttcaaggcagctgaagagcgtggcttcaccgctgttaagcaccagcgtgaggttggcgcaggctacttcgaccagatcgcaaccaccgttgacccgaactcttctaccaccgctttgaagggttccactgaagaaggccagttccacaactag

SEQ ID NO: 13 - DNA, 35 bp, synthetic construct
  source 1..35: mol_type = other DNA
cggtacccggggatccgttctgtggcaattcttgg

SEQ ID NO: 14 - DNA, 32 bp, synthetic construct
  source 1..32: mol_type = other DNA
aatacacagggcgttgccgactgccgtggcaa

SEQ ID NO: 15 - DNA, 33 bp, synthetic construct
  source 1..33: mol_type = other DNA
acggcagtcggcaacgccctgtgtatttggggc

SEQ ID NO: 16 - DNA, 36 bp, synthetic construct
  source 1..36: mol_type = other DNA
atgcctgcaggtcgacaagcaactcgtgcatgccta

SEQ ID NO: 17 - DNA, 34 bp, synthetic construct
  source 1..34: mol_type = other DNA
cggtacccggggatcccttgatgacaaggcttgg

SEQ ID NO: 18 - DNA, 34 bp, synthetic construct
  source 1..34: mol_type = other DNA
gataacacacttgatgaggtcaagattttcaagg

SEQ ID NO: 19 - DNA, 33 bp, synthetic construct
  source 1..33: mol_type = other DNA
tcatcaagtgtgttatcgataaggagcgactca

SEQ ID NO: 20 - DNA, 34 bp, synthetic construct
  source 1..34: mol_type = other DNA
atgcctgcaggtcgactgcagggcttcgggcttg

SEQ ID NO: 21 - DNA, 34 bp, synthetic construct
  source 1..34: mol_type = other DNA
cggtacccggggatccaatgatcgcagctggcgc

SEQ ID NO: 22 - DNA, 35 bp, synthetic construct
  source 1..35: mol_type = other DNA
gggtgatgaactggaacttagcgatctcatctgcc

SEQ ID NO: 23 - DNA, 35 bp, synthetic construct
  source 1..35: mol_type = other DNA
gttccagttcatcaccctcgcaggcttccactccc

SEQ ID NO: 24 - DNA, 35 bp, synthetic construct
  source 1..35: mol_type = other DNA
atgcctgcaggtcgacgacggtgcgggaaatagac